European Patent Application EP 4 450 079 A1, published October 23, 2024. Title: 신규한 펩타이드를 포함하는 황반변성의 치료용 조성물. Applicant: 아이바이오코리아. The sequence listing filed with the application follows.

SEQUENCE LISTING (45 sequences)

SEQ ID NO: 1 - protein, 5 aa, synthetic construct
  REGION 1..5: note = Xaa at position 1 is Trans-4-hydroxy-L-proline.
XGQDV

SEQ ID NO: 2 - protein, 5 aa, synthetic construct
  REGION 1..5: note = Xaa at position 1 is Trans-4-hydroxy-L-proline
XGQDL

SEQ ID NO: 3 - protein, 5 aa, synthetic construct
  REGION 1..5: note = Xaa at position 1 is Trans-4-hydroxy-L-proline.
XGQDA

SEQ ID NO: 4-5 - skipped (2 entries)

SEQ ID NO: 6 - protein, 5 aa, synthetic construct
  REGION 1..5: note = Xaa at position 1 is Trans-4-Hydroxy-D-proline.
XGQDG

SEQ ID NO: 7 - protein, 6 aa, synthetic construct
  REGION 1..6: note = Xaa at position 1 is Trans-4-hydroxy-L-proline.
XGQDVL

SEQ ID NO: 8 - protein, 6 aa, synthetic construct
  REGION 1..6: note = Xaa at position 1 is Trans-4-hydroxy-L-proline.
XGQDLL

SEQ ID NO: 9 - protein, 6 aa, synthetic construct
  REGION 1..6: note = Xaa at position 1 is Trans-4-hydroxy-L-proline.
XGQDAL

SEQ ID NO: 10 - protein, 6 aa, synthetic construct
  REGION 1..6: note = Xaa at position 1 is Trans-4-hydroxy-L-proline. Xaa at position 2is D-Glutamine.
XGXDGL

SEQ ID NO: 11 - protein, 6 aa, synthetic construct
  REGION 1..6: note = Xaa at position 1 is Trans-4-hydroxy-L-proline. Xaa at position 2is D-Aspartate or D-Aspartic acid.
XGQXGL

SEQ ID NO: 12 - protein, 6 aa, synthetic construct
  REGION 1..6: note = Xaa at position 1 is Trans-4-hydroxy-L-proline. Xaa at position 2is D-Leucine.
XGQDGX

SEQ ID NO: 13 - protein, 6 aa, synthetic construct
  REGION 1..6: note = Xaa at position 1 is Trans-4-Hydroxy-D-proline.
XGQDGL

SEQ ID NO: 14 - protein, 7 aa, synthetic construct
  REGION 1..7: note = Xaa at position 1 is Trans-4-hydroxy-L-proline.
XGQDVLA

SEQ ID NO: 15 - protein, 7 aa, synthetic construct
  REGION 1..7: note = Xaa at position 1 is Trans-4-hydroxy-L-proline.
XGQDLLA

SEQ ID NO: 16 - protein, 7 aa, synthetic construct
  REGION 1..7: note = Xaa at position 1 is Trans-4-hydroxy-L-proline.
XGQDALA

SEQ ID NO: 17 - protein, 7 aa, synthetic construct
  REGION 1..7: note = Xaa at position 1 is Trans-4-hydroxy-L-proline. Xaa at position 2is Alanine substituted with isopropyl ester.
XGQDGLX

SEQ ID NO: 18 - protein, 7 aa, synthetic construct
  REGION 1..7: note = Xaa at position 1 is Trans-4-hydroxy-L-proline. Xaa at position 2is D-Glutamine.
XGXDGLA

SEQ ID NO: 19 - protein, 7 aa, synthetic construct
  REGION 1..7: note = Xaa at position 1 is Trans-4-hydroxy-L-proline. Xaa at position 2is D-Aspartate or D-Aspartic acid.
XGQXGLA

SEQ ID NO: 20 - protein, 7 aa, synthetic construct
  REGION 1..7: note = Xaa at position 1 is Trans-4-hydroxy-L-proline. Xaa at position 2is D-Leucine.
XGQDGXA

SEQ ID NO: 21 - protein, 7 aa, synthetic construct
  REGION 1..7: note = Xaa at position 1 is Trans-4-hydroxy-L-proline. Xaa at position 2is D-Alanine.
XGQDGLX

SEQ ID NO: 22 - protein, 5 aa, synthetic construct
  REGION 1..5: note = Xaa at position 1 is Cis-4-fluoro-L-proline.
XGQDG

SEQ ID NO: 23 - protein, 5 aa, synthetic construct
  REGION 1..5: note = Xaa at position 1 is Trans-4-amino-L-proline.
XGQDG

SEQ ID NO: 24 - protein, 5 aa, synthetic construct
  REGION 1..5: note = Xaa at position 1 is 4,4-difluoro-L-proline.
XGQDG

SEQ ID NO: 25 - protein, 5 aa, synthetic construct
  REGION 1..5: note = Xaa at position 1 is 4-methylene-L-proline.
XGQDG

SEQ ID NO: 26 - protein, 5 aa, synthetic construct
  REGION 1..5: note = Xaa at position 1 is 4,4-Dimethyl-L-proline.
XGQDG

SEQ ID NO: 27 - protein, 6 aa, synthetic construct
  REGION 1..6: note = Xaa at position 1 is Cis-4-fluoro-L-proline.
XGQDGL

SEQ ID NO: 28 - protein, 6 aa, synthetic construct
  REGION 1..6: note = Xaa at position 1 is Trans-4-amino-L-proline.
XGQDGL

SEQ ID NO: 29 - protein, 6 aa, synthetic construct
  REGION 1..6: note = Xaa at position 1 is 4,4-difluoro-L-proline.
XGQDGL

SEQ ID NO: 30 - protein, 6 aa, synthetic construct
  REGION 1..6: note = Xaa at position 1 is 4-methylene-L-proline.
XGQDGL

SEQ ID NO: 31 - protein, 6 aa, synthetic construct
  REGION 1..6: note = Xaa at position 1 is 4,4-Dimethyl-L-proline.
XGQDGL

SEQ ID NO: 32 - protein, 7 aa, synthetic construct
  REGION 1..7: note = Xaa at position 1 is Trans-4-Hydroxy-D-proline.
XGQDGLA

SEQ ID NO: 33 - protein, 7 aa, synthetic construct
  REGION 1..7: note = Xaa at position 1 is Cis-4-fluoro-L-proline.
XGQDGLA

SEQ ID NO: 34 - protein, 7 aa, synthetic construct
  REGION 1..7: note = Xaa at position 1 is 4-methylene-L-proline.
XGQDGLA

SEQ ID NO: 35 - protein, 7 aa, synthetic construct
  REGION 1..7: note = Xaa at position 1 is 4-methylene-L-proline.
XGQDGLA

SEQ ID NO: 36 - protein, 5 aa, synthetic construct
  REGION 1..5: note = Xaa at position 1 is Trans-4-hydroxy-L-proline.
XGQEG

SEQ ID NO: 37 - protein, 5 aa, synthetic construct
  REGION 1..5: note = Xaa at position 1 is Trans-4-hydroxy-L-proline.
XGQEV

SEQ ID NO: 38 - protein, 6 aa, synthetic construct
  REGION 1..6: note = Xaa at position 1 is Trans-4-hydroxy-L-proline.
XGQELL

SEQ ID NO: 39 - protein, 6 aa, synthetic construct
  REGION 1..6: note = Xaa at position 1 is Trans-4-hydroxy-L-proline.
XGQEVL

SEQ ID NO: 40 - protein, 7 aa, synthetic construct
  REGION 1..7: note = Xaa at position 1 is Trans-4-hydroxy-L-proline.
XGQEGLA

SEQ ID NO: 41 - protein, 7 aa, synthetic construct
  REGION 1..7: note = Xaa at position 1 is Trans-4-hydroxy-L-proline.
XGQELLA

SEQ ID NO: 42 - protein, 7 aa, synthetic construct
  REGION 1..7: note = Xaa at position 1 is Trans-4-hydroxy-L-proline.
XGQEVLA

SEQ ID NO: 43 - protein, 7 aa, synthetic construct
  REGION 1..7: note = Xaa at position 1 is Trans-4-hydroxy-L-proline. Xaa at position 2is 2-aminoisobutyric acid.
XGQEXLA

SEQ ID NO: 44 - protein, 7 aa, synthetic construct
  REGION 1..7: note = Xaa at position 1 is Trans-4-hydroxy-L-proline. Xaa at position 2is L-alpha-tert-Butylglycine.
XGQEXLA

SEQ ID NO: 45 - protein, 7 aa, synthetic construct
  REGION 1..7: note = Xaa at position 1 is Trans-4-hydroxy-L-proline. Xaa at position 2is Phenylglycine.
XGQEXLA